European Patent Specification EP 2 773 212 B1, published August 7, 2024. Title: Methods and Compositions for Treatment of Autism. Applicant: The Johns Hopkins University Talalay, Paul Zimmerman, Andrew W. Smith, Kirby D. The sequence listing filed with the application follows.

SEQUENCE LISTING (52 sequences)

SEQ ID NO: 1 - DNA, 20 bp, Artificial Sequence
  Description of Artificial Sequence: note = synthetic construct
cccagaaacttggactggaa

SEQ ID NO: 2 - DNA, 20 bp, Artificial Sequence
  Description of Artificial Sequence: note = synthetic construct
cccagcgctaagagtaaacg

SEQ ID NO: 3 - DNA, 20 bp, Artificial Sequence
  Description of Artificial Sequence: note = synthetic construct
caggtggcacagcttaaaca

SEQ ID NO: 4 - DNA, 20 bp, Artificial Sequence
  Description of Artificial Sequence: note = synthetic construct
tgagttggcacccactgtta

SEQ ID NO: 5 - DNA, 20 bp, Artificial Sequence
  Description of Artificial Sequence: note = synthetic construct
agctgctgaagaggcaagag

SEQ ID NO: 6 - DNA, 20 bp, Artificial Sequence
  Description of Artificial Sequence: note = synthetic construct
ctccaggaaaagcaaagctg

SEQ ID NO: 7 - DNA, 20 bp, Artificial Sequence
  Description of Artificial Sequence: note = synthetic construct
tgaagccatggattttgaca

SEQ ID NO: 8 - DNA, 20 bp, Artificial Sequence
  Description of Artificial Sequence: note = synthetic construct
tattggaagggccttgtctg

SEQ ID NO: 9 - DNA, 20 bp, Artificial Sequence
  Description of Artificial Sequence: note = synthetic construct
tatcagacagcgcagtcacc

SEQ ID NO: 10 - DNA, 20 bp, Artificial Sequence
  Description of Artificial Sequence: note = synthetic construct
caatgtcaccacctccacag

SEQ ID NO: 11 - DNA, 20 bp, Artificial Sequence
  Description of Artificial Sequence: note = synthetic construct
ggcagctggttttattggaa

SEQ ID NO: 12 - DNA, 20 bp, Artificial Sequence
  Description of Artificial Sequence: note = synthetic construct
acagtttcacgtccccactc

SEQ ID NO: 13 - DNA, 19 bp, Artificial Sequence
  Description of Artificial Sequence: note = synthetic construct
gcacaggaaaccagttagg

SEQ ID NO: 14 - DNA, 20 bp, Artificial Sequence
  Description of Artificial Sequence: note = synthetic construct
atctgggttttccaaagcaa

SEQ ID NO: 15 - DNA, 20 bp, Artificial Sequence
  Description of Artificial Sequence: note = synthetic construct
agatgacctggaaaccatgc

SEQ ID NO: 16 - DNA, 20 bp, Artificial Sequence
  Description of Artificial Sequence: note = synthetic construct
gtgtcatccaacgtggtcag

SEQ ID NO: 17 - DNA, 20 bp, Artificial Sequence
  Description of Artificial Sequence: note = synthetic construct
actgcctggaggatagcaga

SEQ ID NO: 18 - DNA, 20 bp, Artificial Sequence
  Description of Artificial Sequence: note = synthetic construct
accttggactgctggatgtc

SEQ ID NO: 19 - DNA, 20 bp, Artificial Sequence
  Description of Artificial Sequence: note = synthetic construct
aatgaccagaatcgcctgac

SEQ ID NO: 20 - DNA, 20 bp, Artificial Sequence
  Description of Artificial Sequence: note = synthetic construct
cgctccttgagctttttgtc

SEQ ID NO: 21 - DNA, 20 bp, Artificial Sequence
  Description of Artificial Sequence: note = synthetic construct
ccgctccacagagatacaca

SEQ ID NO: 22 - DNA, 20 bp, Artificial Sequence
  Description of Artificial Sequence: note = synthetic construct
gtcttgtccgtccatccact

SEQ ID NO: 23 - DNA, 20 bp, Artificial Sequence
  Description of Artificial Sequence: note = synthetic construct
gcagaacctcagccactttc

SEQ ID NO: 24 - DNA, 20 bp, Artificial Sequence
  Description of Artificial Sequence: note = synthetic construct
accgaggagacgagactgaa

SEQ ID NO: 25 - DNA, 20 bp, Artificial Sequence
  Description of Artificial Sequence: note = synthetic construct
ggcagaggctgataagaacg

SEQ ID NO: 26 - DNA, 20 bp, Artificial Sequence
  Description of Artificial Sequence: note = synthetic construct
agacaggagcgcagtttcat

SEQ ID NO: 27 - DNA, 20 bp, Artificial Sequence
  Description of Artificial Sequence: note = synthetic construct
ccgagaaggacgagtttgag

SEQ ID NO: 28 - DNA, 20 bp, Artificial Sequence
  Description of Artificial Sequence: note = synthetic construct
ctggtacagtccgctgatga

SEQ ID NO: 29 - DNA, 20 bp, Artificial Sequence
  Description of Artificial Sequence: note = synthetic construct
gatattttgcccagcaggaa

SEQ ID NO: 30 - DNA, 20 bp, Artificial Sequence
  Description of Artificial Sequence: note = synthetic construct
tttgtctcccgttttggaac

SEQ ID NO: 31 - DNA, 19 bp, Artificial Sequence
  Description of Artificial Sequence: note = synthetic construct
acacggtccacagctcatc

SEQ ID NO: 32 - DNA, 22 bp, Artificial Sequence
  Description of Artificial Sequence: note = synthetic construct
tcttgcctccaaagtatgtcaa

SEQ ID NO: 33 - DNA, 20 bp, Artificial Sequence
  Description of Artificial Sequence: note = synthetic construct
tccgatgggtccttacactc

SEQ ID NO: 34 - DNA, 20 bp, Artificial Sequence
  Description of Artificial Sequence: note = synthetic construct
taaggaagccagccaagaga

SEQ ID NO: 35 - DNA, 20 bp, Artificial Sequence
  Description of Artificial Sequence: note = synthetic construct
ccctggaacctcacatcaac

SEQ ID NO: 36 - DNA, 20 bp, Artificial Sequence
  Description of Artificial Sequence: note = synthetic construct
cgttagggctgaggtttgtc

SEQ ID NO: 37 - DNA, 24 bp, Artificial Sequence
  Description of Artificial Sequence: note = synthetic construct
acgttgctatccaggctgtgctat

SEQ ID NO: 38 - DNA, 24 bp, Artificial Sequence
  Description of Artificial Sequence: note = synthetic construct
cggtgaggatcttcatgaggtagt

SEQ ID NO: 39 - DNA, 17 bp, Artificial Sequence
  Description of Artificial Sequence: note = synthetic construct
ttgccgccagaacacag

SEQ ID NO: 40 - DNA, 20 bp, Artificial Sequence
  Description of Artificial Sequence: note = synthetic construct
acttgcccgaatctacgtgt

SEQ ID NO: 41 - DNA, 25 bp, Artificial Sequence
  Description of Artificial Sequence: note = synthetic construct
tgctgtctccatgtttgatgtatct

SEQ ID NO: 42 - DNA, 22 bp, Artificial Sequence
  Description of Artificial Sequence: note = synthetic construct
tctctgctccccacctctaagt

SEQ ID NO: 43 - DNA, 20 bp, Artificial Sequence
  Description of Artificial Sequence: note = synthetic construct
ggagctggaagcctggtatg

SEQ ID NO: 44 - DNA, 18 bp, Artificial Sequence
  Description of Artificial Sequence: note = synthetic construct
gctctgggaggtgcttgt

SEQ ID NO: 45 - DNA, 20 bp, Artificial Sequence
  Description of Artificial Sequence: note = synthetic construct
caagatcctggaccgtgtca

SEQ ID NO: 46 - DNA, 21 bp, Artificial Sequence
  Description of Artificial Sequence: note = synthetic construct
tggccatttctgtggacatca

SEQ ID NO: 47 - DNA, 21 bp, Artificial Sequence
  Description of Artificial Sequence: note = synthetic construct
tgcagaagaaaatggatttcg

SEQ ID NO: 48 - DNA, 19 bp, Artificial Sequence
  Description of Artificial Sequence: note = synthetic construct
actgtccatctgcagccac

SEQ ID NO: 49 - DNA, 20 bp, Artificial Sequence
  Description of Artificial Sequence: note = synthetic construct
gcgatgattctgacatttgg

SEQ ID NO: 50 - DNA, 21 bp, Artificial Sequence
  Description of Artificial Sequence: note = synthetic construct
aatgaagccacagctttatca

SEQ ID NO: 51 - DNA, 19 bp, Artificial Sequence
  Description of Artificial Sequence: note = synthetic construct
ataattcccccaccacctc

SEQ ID NO: 52 - DNA, 25 bp, Artificial Sequence
  Description of Artificial Sequence: note = synthetic construct
caccttccttctttttgattttgtc